European Patent Specification EP 4 185 716 B1, published February 19, 2025. Title: Method for in vitro diagnosis of head and neck cancer and related kit. Applicant: Eurofins Genoma Group Srl Istituti Fisioterapici Ospitalieri. The sequence listing filed with the application follows.

SEQUENCE LISTING (6 sequences)

SEQ ID NO: 1 - DNA, 27 bp, Homo sapiens
gcgcacgtccagccgcgccccggcccg

SEQ ID NO: 2 - DNA, 27 bp, Homo sapiens
gcgcacgtccagccgcgccccggcccg

SEQ ID NO: 3 - DNA, 26 bp, Homo sapiens
cgggccggggcgcggctggacgtgcg

SEQ ID NO: 4 - DNA, 16 bp, Homo sapiens
tagtggatggtggtac

SEQ ID NO: 5 - DNA, 16 bp, Homo sapiens
tagtggatggtggtac

SEQ ID NO: 6 - DNA, 15 bp, Homo sapiens
gtaccaccatccact